European Patent Application EP 4 202 394 A1, published June 28, 2023. Title: USE OF A SHRINKABLE BIOPOLYMER FIBER AS SENSOR. Applicant: AMSilk GmbH. Application EP. The sequence listing filed with the application follows.

SEQUENCE LISTING (7 sequences)

SEQ ID NO: 1 - protein, 35 aa, synthetic construct
  REGION 1..35: note = synthetic
  DOMAIN 1..35: note = Module C (ADF-4)
GSSAAAAAAAASGPGGYGPENQGPSGPGGYGPGGP

SEQ ID NO: 2 - protein, 35 aa, synthetic construct
  REGION 1..35: note = synthetic
  DOMAIN 1..35: note = Module Cc
GSSAAAAAAAASGPGGYGPENQGPCGPGGYGPGGP

SEQ ID NO: 3 - protein, 35 aa, synthetic construct
  REGION 1..35: note = synthetic
  DOMAIN 1..35: note = C kappa
GSSAAAAAAAASGPGGYGPKNQGPSGPGGYGPGGP

SEQ ID NO: 4 - protein, 124 aa, synthetic construct
  REGION 1..124: note = based on ADF-3
  DOMAIN 1..124: note = NR3 (ADF-3)
GAASAAVSVGGYGPQSSSAPVASAAASRLSSPAASSRVSSAVSSLVSSGPTNQAALSNTISSVVSQVSASNPGLSGCDVLVQALLEVVSALVSILGSSSIGQINYGASAQYTQMVGQSVAQALA

SEQ ID NO: 5 - protein, 109 aa, synthetic construct
  REGION 1..109: note = based on ADF-4
  DOMAIN 1..109: note = NR4 (ADF-4)
GAYGPSPSASASVAASRLSSPAASSRVSSAVSSLVSSGPTNGAAVSGALNSLVSQISASNPGLSGCDALVQALLELVSALVAILSSASIGQVNVSSVSQSTQMISQALS

SEQ ID NO: 6 - protein, 136 aa, synthetic construct
  REGION 1..136: note = synthetic
  REGION 1..136: note = domain - derived from Latrodectus hesperus (NR5)
MGQANTPWSSKANADAFINSFISAASNTGSFSQDQMEDMSLIGNTLMAAMDNMGGRITPSKLQALDMAFASSVAEIAASEGGDLGVTTNAIADALTSAFYQTTGVVNSRFISEIRSLIGMFAQASANDVYASAGSG

SEQ ID NO: 7 - protein, 137 aa, synthetic construct
  REGION 1..137: note = synthetic
  REGION 1..137: note = domain - derived from Latrodectus hesperus (NR6)
MGQANTPWSSKENADAFIGAFMNAASQSGAFSSDQIDDMSVISNTLMAAMDNMGGRITQSKLQALDMAFASSVAEIAVADGQNVGAATNAISDALRSAFYQTTGVVNNQFITGISSLIGMFAQVSGNEVSYSSAGSG